European Patent Specification EP 4 210 720 B1, published August 21, 2024. Title: Probiotic compositions for the treatment of acne. Applicant: Bionou Research S.L. The sequence listing filed with the application follows.

SEQUENCE LISTING (1 sequence)

SEQ ID NO: 1 - RNA, 1558 nt, Lactobacillus rhamnosus
  16s rRNA sequence
agagtttgatcctggctcaggatgaacgctggcggcgtgcctaatacatgcaagtcgaacgagttctgattattgaaaggtgcttgcatcttgatttaattttgaacgagtggcggacgggtgagtaacacgtgggtaacctgcccttaagtgggggataacatttggaaacagatgctaataccgcataaatccaagaaccgcatggttcttggctgaaagatggcgtaagctatcgcttttggatggacccgcggcgtattagctagttggtgaggtaacggctcaccaaggcaatgatacgtagccgaactgagaggttgatcggccacattgggactgagacacggcccaaactcctacgggaggcagcagtagggaatcttccacaatggacgcaagtctgatggagcaacgccgcgtgagtgaagaaggctttcgggtcgtaaaactctgttgttggagaagaatggtcggcagagtaactgttgtcggcgtgacggtatccaaccagaaagccacggctaactacgtgccagcagccgcggtaatacgtaggtggcaagcgttatccggatttattgggcgtaaagcgagcgcaggcggttttttaagtctgatgtgaaagccctcggcttaaccgaggaagtgcatcggaaactggaaaacttgagtgcagaagaggacagtggaactccatgtgtagcggtgaaatgcgtagatatatggaagaacaccagtggcgaaggcggctgtctggtctgtaactgacgctgaggctcgaaagcatgggtagcgaacaggattagataccctggtagtccatgccgtaaacgatgaatgctaggtgttggagggtttccgcccttcagtgccgcagctaacgcattaagcattccgcctggggagtacgaccgcaaggttgaaactcaaaggaattgacgggggcccgcacaagcggtggagcatgtggtttaattcgaagcaacgcgaagaaccttaccaggtcttgacatcttttgatcacctgagagatcgggtttccccttcgggggcaaaatgacaggtggtgcatggttgtcgtcagctcgtgtcgtgagatgttgggttaagtcccgcaacgagcgcaacccttatgactagttgccagcatttagttgggcactctagtaagactgccggtgacaaaccggaggaaggtggggatgacgtcaaatcatcatgccccttatgacctgggctacacacgtgctacaatggatggtacaacgagttgcgagaccgcgaggtcaagctaatctcttaaagccattctcagttcggactgtaggctgcaactcgcctacacgaagtcggaatcgctagtaatcgcggatcagcacgccgcggtgaatacgttcccgggccttgtacacaccgcccgtcacaccatgagagtttgtaacacccgaagccggtggcgtaacccttttagggagcgagccgtctaaggtgggacaaatgattagggtgaagtcgtaacaaggtagccgtaggagaacctgcggctggatcacct